European Patent Application EP 4 692 109 A1, published February 11, 2026. Title: 濾胞性ヘルパーＴ細胞誘導性ＳＡＲＳ－ＣｏＶ－２スパイクタンパク質の部分ペプチド. Applicant: 国立大学法人大阪大学. The sequence listing filed with the application follows.

SEQUENCE LISTING (70 sequences)

SEQ ID NO: 1 - protein, 11 aa, SARS-CoV-2
FKIYSKHTPIN

SEQ ID NO: 2 - protein, 15 aa, SARS-CoV-2
FQFCNDPFLGVYYHK

SEQ ID NO: 3 - protein, 11 aa, SARS-CoV-2
KRFDNPVLPFN

SEQ ID NO: 4 - protein, 11 aa, SARS-CoV-2
LLQYGSFCTQL

SEQ ID NO: 5 - protein, 15 aa, SARS-CoV-2
PPAYTNSFTRGVYYP

SEQ ID NO: 6 - protein, 15 aa, SARS-CoV-2
CSNLLLQYGSFCTQL

SEQ ID NO: 7 - protein, 15 aa, SARS-CoV-2
SKRSFIEDLLFNKVT

SEQ ID NO: 8 - protein, 15 aa, SARS-CoV-2
TGVLTESNKKFLPFQ

SEQ ID NO: 9 - protein, 15 aa, SARS-CoV-2
TNGTKRFDNPVLPFN

SEQ ID NO: 10 - protein, 11 aa, SARS-CoV-2
NQFNSAIGKIQ

SEQ ID NO: 11 - protein, 11 aa, SARS-CoV-2
NFTISVTTEIL

SEQ ID NO: 12 - protein, 15 aa, SARS-CoV-2
STEIYQAGSTPCNGV

SEQ ID NO: 13 - protein, 11 aa, SARS-CoV-2
KVFRSSVLHST

SEQ ID NO: 14 - protein, 11 aa, SARS-CoV-2
EIRASANLAAT

SEQ ID NO: 15 - protein, 15 aa, SARS-CoV-2
NFTISVTTEILPVSM

SEQ ID NO: 16 - protein, 15 aa, SARS-CoV-2
FIKQYGDCLGDIAAR

SEQ ID NO: 17 - protein, 15 aa, SARS-CoV-2
FIEDLLFNKVTLADA

SEQ ID NO: 18 - protein, 13 aa, Homo sapiens
CAVLNQAGTALIF

SEQ ID NO: 19 - protein, 13 aa, Homo sapiens
CASSGRPEGPQHF

SEQ ID NO: 20 - protein, 14 aa, Homo sapiens
CAESRYMGRRALTF

SEQ ID NO: 21 - protein, 12 aa, Homo sapiens
CASSLEGTEAFF

SEQ ID NO: 22 - protein, 14 aa, Homo sapiens
CAGAGGTSYGKLTF

SEQ ID NO: 23 - protein, 11 aa, Homo sapiens
CASSLLGEQYF

SEQ ID NO: 24 - protein, 14 aa, Homo sapiens
CVVNKGSSASKIIF

SEQ ID NO: 25 - protein, 14 aa, Homo sapiens
CASSEGASNQPQHF

SEQ ID NO: 26 - protein, 14 aa, Homo sapiens
CALSMNTGFQKLVF

SEQ ID NO: 27 - protein, 12 aa, Homo sapiens
CSAYSIYNEQFF

SEQ ID NO: 28 - protein, 13 aa, Homo sapiens
CVVSIGFGNVLHC

SEQ ID NO: 29 - protein, 15 aa, Homo sapiens
CASRPNRGDNSPLHF

SEQ ID NO: 30 - protein, 17 aa, Homo sapiens
CAVRRGGSGGSNYKLTF

SEQ ID NO: 31 - protein, 14 aa, Homo sapiens
CASSLMGGAYGYTF

SEQ ID NO: 32 - protein, 14 aa, Homo sapiens
CLVGPYNQGGKLIF

SEQ ID NO: 33 - protein, 14 aa, Homo sapiens
CSARDVEVGSGYTF

SEQ ID NO: 34 - protein, 13 aa, Homo sapiens
CVVGTDSWGKLQF

SEQ ID NO: 35 - protein, 15 aa, Homo sapiens
CASSPLSGSSYEQYF

SEQ ID NO: 36 - protein, 13 aa, Homo sapiens
CALTSAAGNKLTF

SEQ ID NO: 37 - protein, 13 aa, Homo sapiens
CSAIAGDADTQYF

SEQ ID NO: 38 - protein, 14 aa, Homo sapiens
CVVSERASSYKLIF

SEQ ID NO: 39 - protein, 14 aa, Homo sapiens
CAWNLGGGNQPQHF

SEQ ID NO: 40 - protein, 15 aa, Homo sapiens
CLVGDSDTGRRALTF

SEQ ID NO: 41 - protein, 14 aa, Homo sapiens
CASSQGQGSYGYTF

SEQ ID NO: 42 - protein, 14 aa, Homo sapiens
CAVKRGNQGGKLIF

SEQ ID NO: 43 - protein, 13 aa, Homo sapiens
CASGTGSYNEQFF

SEQ ID NO: 44 - protein, 13 aa, Homo sapiens
CAVGIRGNEKLTF

SEQ ID NO: 45 - protein, 16 aa, Homo sapiens
CASSYSGGTVTGELFF

SEQ ID NO: 46 - protein, 15 aa, Homo sapiens
CATNAGGTSYGKLTF

SEQ ID NO: 47 - protein, 16 aa, Homo sapiens
CSARDGQTATNEKLFF

SEQ ID NO: 48 - protein, 14 aa, Homo sapiens
CALGSTSNTGKLIF

SEQ ID NO: 49 - protein, 13 aa, Homo sapiens
CAWSVKGFPSQHF

SEQ ID NO: 50 - protein, 14 aa, Homo sapiens
CAGAKGSGTYKYIF

SEQ ID NO: 51 - protein, 15 aa, Homo sapiens
CASSSRTGYNSPLHF

SEQ ID NO: 52 - protein, 15 aa, Homo sapiens
CVVNMVTGGYNKLIF

SEQ ID NO: 53 - protein, 13 aa, Homo sapiens
CASSSDRNYGYTF

SEQ ID NO: 54 - protein, 19 aa, Homo sapiens
CASSYPPSGGRTGFGEAFF

SEQ ID NO: 55 - protein, 14 aa, Homo sapiens
CAMRDIGFGNVLHC

SEQ ID NO: 56 - protein, 14 aa, Homo sapiens
CAASIPNSGYALNF

SEQ ID NO: 57 - protein, 14 aa, Homo sapiens
CSASIEQGDLGYTF

SEQ ID NO: 58 - protein, 16 aa, Homo sapiens
CAVNEYSGAGSYQLTF

SEQ ID NO: 59 - protein, 18 aa, Homo sapiens
CASSVGQSKGKSAETQYF

SEQ ID NO: 60 - protein, 13 aa, Homo sapiens
CALSDGAGNKLTF

SEQ ID NO: 61 - protein, 14 aa, Homo sapiens
CSAGDTASTYGYTF

SEQ ID NO: 62 - protein, 15 aa, Homo sapiens
CAFMKQRGGSEKLVF

SEQ ID NO: 63 - protein, 13 aa, Homo sapiens
CAWSLQGQRPQHF

SEQ ID NO: 64 - protein, 15 aa, Homo sapiens
DGYFKIYSKHTPINL

SEQ ID NO: 65 - protein, 15 aa, Homo sapiens
TNGTKRFDNPVLPFN

SEQ ID NO: 66 - protein, 15 aa, Homo sapiens
CSNLLLQYGSFCTQL

SEQ ID NO: 67 - protein, 15 aa, Homo sapiens
KVFRSSVLHSTQDLF

SEQ ID NO: 68 - protein, 15 aa, Homo sapiens
EIRASANLAATKMSE

SEQ ID NO: 69 - protein, 15 aa, SARS-CoV-2
DGYFKIYSKHTPINL

SEQ ID NO: 70 - protein, 14 aa, SARS-CoV-2
EMIAQYTSALLAGT